European Patent Application EP 4 643 886 A1, published November 5, 2025. Title: ANTI-CD33/CLL1 BISPECIFIC ANTIBODY-NATURAL KILLER CELL CONJUGATE AND USE THEREOF. Applicant: IMBIORAY (HANGZHOU) BIOMEDICINE CO., LTD. The sequence listing filed with the application follows.

SEQUENCE LISTING (20 sequences)

SEQ ID NO: 1 - protein, 118 aa, synthetic construct
QVQLQESGPGLVKPSETLSLTCVVSGGSISSSNWWSWVRQPPGKGLEWIGEIYHSGSPDYNPSLKSRVTISVDKSRNQFSLKLSSVTAADTAVYYCAKVSTGGFFDYWGQGTLVTVSS

SEQ ID NO: 2 - protein, 330 aa, synthetic construct
ASTKGPSVFPLAPSSKSTSGGTAALGCLVKDYFPEPVTVSWNSGALTSGVHTFPAVLQSSGLYSLSSVVTVPSSSLGTQTYICNVNHKPSNTKVDKRVEPKSCDKTHTSPPCPAPELLGGPSVFLFPPKPKDTLMISRTPEVTCVVVDVSHEDPEVKFNWYVDGVEVHNAKTKPREEQYNSTYRVVSVLTVLHQDWLNGKEYKCKVSNKALPAPIEKTISKAKGQPREPQVYTLPPSREEMTKNQVSLTCLVKGFYPSDIAVEWESNGQPENNYKTTPPVLDSDGSFFLYSRLTVDKSRWQQGNVFSCSVMHEALHNHYTQKSLSLSPGK

SEQ ID NO: 3 - protein, 111 aa, synthetic construct
DIQMTQSPSSLSASVGDRVTITCRASQSISSYLNWYQQKPGKAPKLLIYAASSLQSGVPSRFSGSGSGTDFTLTISSLQPEDFATYYCQQSYSTPPTFGQGTKVEIKRTVA

SEQ ID NO: 4 - protein, 103 aa, synthetic construct
APSVFIFPPSDEQLKSGTASVVCLLNNFYPREAKVQWKVDNALQSGNSQESVTEQDSKDSTYSLSSTLTLSKADYEKHKVYACEVTHQGLSSPVTKSFNRGEC

SEQ ID NO: 5 - protein, 116 aa, synthetic construct
QVQLVQSGAEVKKPGSSVKVSCKASGYTFTDYNMHWVRQAPGQGLEWIGYIYPYNGGTGYNQKFKSKATITADESTNTAYMELSSLRSEDTAVYYCARGRPAMDYWGQGTLVTVSS

SEQ ID NO: 6 - protein, 330 aa, synthetic construct
ASTKGPSVFPLAPSSKSTSGGTAALGCLVKDYFPEPVTVSWNSGALTSGVHTFPAVLQSSGLYSLSSVVTVPSSSLGTQTYICNVNHKPSNTKVDKRVEPKSCDKTHTSPPCPAPELLGGPSVFLFPPKPKDTLMISRTPEVTCVVVDVSHEDPEVKFNWYVDGVEVHNAKTKPREEQYNSTYRVVSVLTVLHQDWLNGKEYKCKVSNKALPAPIEKTISKAKGQPREPQVYTLPPSREEMTKNQVSLTCLVKGFYPSDIAVEWESNGQPENNYKTTPPVLDSDGSFLLYSKLTVDKSRWQQGNVFSCSVMHEALHNHYTQKSLSLSPGK

SEQ ID NO: 7 - protein, 115 aa, synthetic construct
DIQMTQSPSSLSASVGDRVTITCRASESVDNYGISFMNWFQQKPGKAPKLLIYAASNQGSGVPSRFSGSGSGTDFTLTISSLQPDDFATYYCQQSKEVPWTFGQGTKVEIKRTVA

SEQ ID NO: 8 - protein, 103 aa, synthetic construct; identical to SEQ ID NO: 4

SEQ ID NO: 9 - protein, 5 aa, synthetic construct
DYNMH

SEQ ID NO: 10 - protein, 17 aa, synthetic construct
YIYPYNGGTGYNQKFKS

SEQ ID NO: 11 - protein, 7 aa, synthetic construct
GRPAMDY

SEQ ID NO: 12 - protein, 15 aa, synthetic construct
RASESVDNYGISFMN

SEQ ID NO: 13 - protein, 7 aa, synthetic construct
AASNQGS

SEQ ID NO: 14 - protein, 8 aa, synthetic construct
QQSKEVPW

SEQ ID NO: 15 - protein, 6 aa, synthetic construct
SSNWWS

SEQ ID NO: 16 - protein, 16 aa, synthetic construct
EIYHSGSPDYNPSLKS

SEQ ID NO: 17 - protein, 9 aa, synthetic construct
VSTGGFFDY

SEQ ID NO: 18 - protein, 11 aa, synthetic construct
RASQSISSYLN

SEQ ID NO: 19 - protein, 7 aa, synthetic construct
AASSLQS

SEQ ID NO: 20 - protein, 9 aa, synthetic construct
QQSYSTPPT